European Patent Specification EP 3 565 638 B1, published March 6, 2024. Title: COMPOUNDS FOR TREATING CANCER. Applicant: BICYCLE THERAPEUTICS LIMITED. The sequence listing filed with the application follows.

SEQUENCE LISTING (17 sequences)

SEQ ID NO: 1 - protein, 13 aa, Artificial Sequence
  source: /note="Description of Artificial Sequence: Synthetic peptide"
  MOD_RES (2)..(2): Any amino acid
  MOD_RES (3)..(3): /replace="Cys" or "Gln" or "Met" or "Ser" or "Thr" or "Gly" or "Ala" or "Ile" or "Leu" or "Pro" or "Val"
  MOD_RES (4)..(5): Any amino acid
  MOD_RES (11)..(12): Any amino acid
  source: /note="See specification as filed for detailed description of substitutions and preferred embodiments"
CXNXXGEDFYXXC

SEQ ID NO: 2 - protein, 14 aa, Artificial Sequence
  source: /note="Description of Artificial Sequence: Synthetic peptide"
CYNEFGCEDFYDIC

SEQ ID NO: 3 - protein, 14 aa, Artificial Sequence
  source: /note="Description of Artificial Sequence: Synthetic peptide"
CYNEFGCEDFYDIC

SEQ ID NO: 4 - protein, 14 aa, Artificial Sequence
  source: /note="Description of Artificial Sequence: Synthetic peptide"
  MOD_RES (2)..(2): D-Ala
CXNEFGCEDFYDIC

SEQ ID NO: 5 - protein, 14 aa, Artificial Sequence
  source: /note="Description of Artificial Sequence: Synthetic peptide"
  MOD_RES (2)..(2): D-Ala
  MOD_RES (5)..(5): 1Nal
  MOD_RES (6)..(6): D-Ala
  MOD_RES (13)..(13): tBuGly
CXNEXXCEDFYDXC

SEQ ID NO: 6 - protein, 14 aa, Artificial Sequence
  source: /note="Description of Artificial Sequence: Synthetic peptide"
  MOD_RES (2)..(2): /replace="Met" or "Phe" or "Val"
  MOD_RES (3)..(3): /replace="Cys" or "Gln" or "Met" or "Ser" or "Thr" or "Gly" or "Ala" or "Ile" or "Leu" or "Pro" or "Val"
  MOD_RES (4)..(4): /replace="Cys" or "Gln" or "Met" or "Ser" or "Thr" or "Asp" or "Glu"
  MOD_RES (5)..(5): /replace="Trp" or "Tyr"
  MOD_RES (12)..(12): /replace="Glu"
  MOD_RES (13)..(13): /replace="Ala" or "Ile" or "Leu" or "Pro" or "Val"
  source: /note="See specification as filed for detailed description of substitutions and preferred embodiments"
CYNNFGCEDFYDGC

SEQ ID NO: 7 - protein, 14 aa, Artificial Sequence
  source: /note="Description of Artificial Sequence: Synthetic peptide"
  MOD_RES (2)..(2): /replace="Met" or "Phe" or "Val"
  MOD_RES (3)..(3): /replace="Gly"
  MOD_RES (4)..(4): /replace="Gln"
CYNEFGCEDFYDIC

SEQ ID NO: 8 - protein, 14 aa, Artificial Sequence
  source: /note="Description of Artificial Sequence: Synthetic peptide"
  MOD_RES (2)..(2): /replace="Met" or "Phe"
  MOD_RES (3)..(3): /replace="Gly"
  MOD_RES (4)..(4): /replace="Gln"
CYNEFGCEDFYDIC

SEQ ID NO: 9 - protein, 14 aa, Artificial Sequence
  source: /note="Description of Artificial Sequence: Synthetic peptide"
  MOD_RES (2)..(2): /replace="Met"
  MOD_RES (4)..(4): /replace="Gln"
CYNEFGCEDFYDIC

SEQ ID NO: 10 - protein, 14 aa, Artificial Sequence
  source: /note="Description of Artificial Sequence: Synthetic peptide"
CMNQFGCEDFYDIC

SEQ ID NO: 11 - protein, 14 aa, Artificial Sequence
  source: /note="Description of Artificial Sequence: Synthetic peptide"
CFGEFGCEDFYDIC

SEQ ID NO: 12 - protein, 14 aa, Artificial Sequence
  source: /note="Description of Artificial Sequence: Synthetic peptide"
CVNEFGCEDFYDIC

SEQ ID NO: 13 - protein, 14 aa, Artificial Sequence
  source: /note="Description of Artificial Sequence: Synthetic peptide"
CFNEFGCEDFYDIC

SEQ ID NO: 14 - protein, 14 aa, Artificial Sequence
  source: /note="Description of Artificial Sequence: Synthetic peptide"
CYNEYGCEDFYDIC

SEQ ID NO: 15 - protein, 14 aa, Artificial Sequence
  source: /note="Description of Artificial Sequence: Synthetic peptide"
CYNEWGCEDFYDIC

SEQ ID NO: 16 - protein, 15 aa, Artificial Sequence
  source: /note="Description of Artificial Sequence: Synthetic peptide"
CKNRGFGCEDFYDIC

SEQ ID NO: 17 - protein, 24 aa, Artificial Sequence
  source: /note="Description of Artificial Sequence: Synthetic peptide"
  MOD_RES (1)..(1): B-Ala
  MOD_RES (2)..(11): Sarcosine
XXXXXXXXXXXACVPCADFPIWYC